European Patent Application EP 4 293 044 A1, published December 20, 2023. Title: ANTI-TRPV6 MONOCLONAL ANTIBODY AND APPLICATION THEREOF. Applicant: COHERENT BIOPHARMA (SUZHOU) , LIMITED. The sequence listing filed with the application follows.

SEQUENCE LISTING (35 sequences)

SEQ ID NO: 1 - DNA, 14538 bp, Homo sapiens
  DNA encoding TRPV6 (1)..(14538)
agagtcctggctggctctgccaagtgtaacaaactcacagccctctccaaactggctggggctgctgggagactcccaaggaactcgtcaggaaggcaggagacaggagacgggacctctacagggagacggtgggccggcccttgggggggctgatgtggccccaaggctgagtcccgtcagggtctggcctcggcctcaggcccccaaggagccggccctacaccccatgggtttgtcactgcccaaggagaaagggctaattctctgcctatggagcaagttctgcagatggttccagagacgggagtcctgggcccagagccgagatgagcagaacctgctgcagcagaagaggtaaggcccccttggtctgctcccttccccacctccccaggcctgcacctctacccctcacccctccctcacctcccgtctttgtttggcacctttggctggacagatggtgctcccaggcccggactggctccttgggagcattctgtcttaagagcctcagcctgtagggctggtgaaagaggatggggttgagatgggcacaggtgttcactatcttaagatctaattcgattctgcaagcctcttgtgagtacttctctaagggccaggcgtcttgctggggcttgtaaggatagagcatcacagcccctccacccaagaggggacggcaggtgaggacaatgccttctgtatctccactgcttgcctctagaacagtctctctggcaggaacacatagtatacatatgttcgcatggaggaatgagtgaacgattgaatgaatgaagcagagagaaccgcggacaccaggaaccagaaaataagacaaaatgtgaaaaaagtgaccattcctatgtatctgtctcatcagacactgaccaaggccttactatttgcccagcactggggggatatgaagacctacaacgctcaaacccaaccttgaggtgtatttctctctcagtgcgggtggggactgaggggaagcgggtcaaaataacagatgttccgaggacctgtgctcttccgcattcaggtggtggaaatcgagactctagcgtttaagccctaaggacattcactggtggcttccagcccctgaaaacttcctaaacccgtgtcctgctttcttcaccatgacagcttggagtacagagcaggagaggagcagggaatcggaactcagggctatccctgcatgtggtctcttcttcaaggtctctaatagagttctctacccagttggtggcatgctagaaggaagtcctgcctgttggggctttccctgggtcacgaaggaggcagatgtctggtcatagaggaaagcctgaagtctttgtgccttagggtttttctctgaccccaagagtaggagcctgctttagcctgaccggggaggctgcctggaggcccctgtgttttcttttgctgaaggattctgggttggggatggtctctttctgtgaattatggcttcccatctctccagccgcccacctctcccccaaggcctgggagagtggggactggagcacatgtttggctgatgacatcttggggcaacagaatggcattgttgttagagagtaggtcgtcctcactggcttcactcatcctcttcccactcttaggaccccagggccaggggatccaggcacagagtgcaaaaaggcctgggggattggaaggggtggtggagattccctgtgtgcgatatcaggggagagcagaggggaggccctgcgctgagtggctgagaataggctgcttccgcatgtcctgtctgccctcacttttcctcagatcatatgggggctgcctctgcagactttggctagaaaggcttgatgtcacccttgggagggatcccccctccctgccctgatctccttactggcctccgcactttcttggccttcttcttgctggatatcaggtgtccagagcaatgactcttctttgggtgggcacttcccagaaggatgctgaaattgcctgcaaggggagtttcctaatctgtgccgtcaaccaaagagaaggcatgggggcattgagataaacatgggatgactaagtaaataggaacaatatggacaagtgaggggtgagctaatggaagaaaggagcacacaatgattgagaacccagtgctgtactaggtactaccacctgccttatctccgtcatcccggtaacaataatggaaggtgggtcctgttatccccctatgaatggggcaggcccagaaccctagagcaagtaaatggtgaagttgaatttgttccaaaggggactcacagggagaactgtggggtgggattgcgtgggattccatgcggtacaggatggtctagtgagaaaggaaggctttgagtctctccaggatgatcgggaacccaaactcctctttttacagtggacgtttcttggtgcttagcacgcagcccgctctgcttaaatctacattgctgggatccaagtcgagctctcaactttctcccgtgtcctccaggtcatctcccccttgggcttgggttttctcacttcctgatatttaatgcattacacatttattgaacataaggcactccacctttctgcagaaaatgaatatgacactgttcctgctctcagggagttctcattcctatgaccaaagtttactgaaggcacatacggggctaaagatgggcttagtagacatcactagaagggtgtaaatgagtgttctggaagcatagagggggaagtgtgagatctgatttcggctgctgtggggtgtcctgggcagcttcatagaggctgcttaacctgaaccccactccagcccatgtgctggcactttgtcatctaaggagcaatttggagggaaggtgatgcttgttggagctttttttagggttaaatacctgtatgaaatgtgtgaattgagtgtctgaaaagtcatccctgggtttctctggtatattgtgcacgcttgccttggtaaatacttacacacatgcctacttgtaaatgcgcaaatagacatgtgcacaaaaggagctgtggcacttaggatggcagccgattccaaatctctaaacaaccactttggctttctcatccccattgccaggaacatgagctggagggaggtggcccacaagtgcccaatgtatgcctccgccccacacattaccgctctttccttcatctgtggtcactgctcaggcttgccccccaacctccaagaaaaatcaggaggagccataaaactagaagaaccacataatttagtggtcagagcctggggctggattcttggccaagcatcctgcctttaactccgtgtgatcttctggcaatgatttggttatgccgcttcagtttccttttctgaagcatgggagaactattcagctggtgttagaaggttgtaaagagcaaaagtgataatgagtgagatgctgcgggaatgagaggggccatgaacttcccctgcacagcactgtatccacccaggaatgcaagaagccacgcactccgagcaaccctgttatgtaccagccccagccctgcccagagggtacactcactggtgggaaaggtatttgtggagagaccagtgggacccatgcctgtcttctctaactcctcttccagccctgattaaaactgagaatcgtgaccaagaaatgaccagtggggcatgcgtcgtggctctgtctctgacttgcttcctccatctgtttcatgagcagatttgactcagtttctgaggggctttctagctctaaaaatcttatttgaacttttctcaagagtcttgtgatcctgccttgtttctcagcacctaaaaaccaaattggacccatgcacacagtgcacacatctacaaggatggaggagcagatgagggtgtggggcggaggagacggagagaggaagtcaggaatccttccctggtggcccagaggcagccctgagaaggaggtcattgatctgtttgctcaagaaataatgtgctagattttgtgccaggaaccccttagttgggttttcaccaggctaatgttgaactagaccgttcaattttattataattaattgcctagtaaaagaaaacattctagaacctgaaaatacctttcatattgttacagtttcagatttgctctataatctcttttgactacttcatcagtgggagcttaaaaggcttcatctgacttttttttgtttctcccttagttgagtatttagtgatccataagaaaacatttttatgtataggatatttctgattccttttcgagtgaagaatcctcattctaaaacggattatgaatcattgtacctctgaatcaggggttctccaccttggactattgacattttggacaggataattctttgcagtgagggctgtcatgtgcagggtgcttagccgtgtccctgcctttgacccccgtgttgtgatctaaactcctgtgataagttgctattgaaaaatctatttgtcccccaagcacaggaatctttgagtaggtcagctctgtgcacctccttcagggacccaaggagagtcaggtgttttggggtcagccttactcccaagcaggtgagctagggctttctgtgctgtccccttgtgggcatatgaggttattgcaagtaatggctgggccggataccttcaaaacccgtccacaggctgggcccccctttttgctggagtctggagttcacagtcggaggaggctagttctctacaaaccttgctgggttgggtcataagctggctcttcacgcagggtgtggtctggctaggttgccagataaaatgcaggacactcagttcaatttaaatttgagataacgaataggctgctagtataagtgtatccccaatattgcacgtgacatacttatactaaaaaaaaattgtgcatctgacattcaaatctaactgagcatcctgtatttttatttggtaactctagcaactctgggtctgacagtagctttttgttttccccaggccactagagtgtcagaattcatagggaatggaggtttatgggggacactttcagcttcagagacgtgtagggaccaaaggggaatctttgagcctgccactgactataccaccactaacatctaggatacagcgagtagaactctggacttggaaaaggtgctctctcggacccatttctagatttgccatcaatctttcacacatttggtcaaaatgggacacaaacgtggaagcatattggaggagggcagggaagagttagtggctggtctcttccctcgagtacccttagcatagaggaagggacacagatacatagcaattacagcacccagtgaaagatgctgaaataaaagtaaggccacaggagagagtgaagaacttctgagtgtctgtgtgtgtgtatgtggtgctagcgattgttttcccctcagtctagggtatctagagaggagggctttgtgcaaatggttgatgtggtggtggtgatggagggaatgtggaaaacttgttttgaagctgtgtttgcataccaagtgtactatttttcacttatatgcttgctgaaagttggcttagcgggcagctgatgaaaataataataacagttaattcaaaccaccttttggcattgctgctgattcattcactctacagatggtgtcagtgagcatctacaccatcctaggtgtatttctaggcataggcagtgcagaagacacaatgaacaattggcgggctgggggagttggattctagaaggaaagagcttcatgggcacagacatagggagaatggtgtgctctgcagtgctgagacaggatgagaccaaaatgccaggtctaaggagtgggtgggacgtgcagagggtggaaaagtagttgcacaaagaccttaaagagcttctgtgttccttatccttagcattttgctaatctgggctagagaatgaagacttgaattaatgagggttagcaggagcaaggaggtagggactgaatgaagagagagctttccatgctgaactgacaggacctggtggcagctgctgtgcatgggggcaaggcagaggagatgagtgagctgatgtctcctctctgattgccctcccacctccagctctggagtcaatttcttgccactgccagcgctttagaatgtgagctcctgtctatgtctttttgtatgtcacataattgtcaaactatggataaatagagttatttcatttactcccatagaaagaccaaatggctccaggccaagagaaaattgaatcaaagggacccatgtgtcttagttggggtaagttctaattttaaaagagatttttagcacacagtaggtataagaataaagagatgatctggggattcagagaagataattttgcctaaaacaagcgagaagtggataataaggagagactaatctgactcagcaaaataaacggatccatgaatcccaaattgggtaaatccaggaagggtccgaagacagaatgggaacattcagatgcacatgaaattcgatgaatgaatcctctagattggattctcttttttctctgcatctgtcattgttggccatagtttgtgtcttaggggccaatagccgaaacaaagtagtatctaaagccctctagacagctggtctgaaaatgatggagaacactgtttcgcaaactttaatgtgagctgtttggaaactgagacccctgagcttgtctctgatttatcgccaccggtttttgcatgcaaggaccacttaagcaatgcttctccaactttcatatgcccaggaatcagctggaaatcttcttaaactgcagatttggattcactaggtggaagggtccgccagagcatttccatttcttataagggctcatgtgctgctgctgatccaggggtccactttaagaaggaaggctgttgagatgatgtgagaagaaagacgagaggcagaaaggaagagacagagataatgaatgaatgaatgaatgaatgaatgaatgaacacctatgaggaaggaaggcctggagccaggcttgttcttatggtccactgttcttttgtgttaagccctgaagatgctattgttgggagggaagcgccaggatcaaagggttctgctgagaaggttgagtaggcagaggatggtgcaacaggagaaatcctgctagcctgtgcatatgactccctccacaaatatgagacaggaattccttgcacccctcggtccatgcaaaacaaggcttatcctggagggcaatctcagggcacctggtgagggtcaaacaggaccactccaggggtaaactggttagcaggtaagcacatgtctacatagaactcctcccctccgtacctgaaatgcactgataatacattcacacatgatacattctggtcccaggacccggtaggggggaaggaaaccagtcacggacaatctcaaaacgcatgctaaatgggcaaaaagttgattgtatttactgactgtaaagagaaaagacatcaatggccccacctgccttgattgaagaccctgaggttcctgctgctgaggcacacacatctgtgtataataatggagtcaagccagggcctctccctccacaactaggtatgctcactgtttccagctttcctattccatcccttcataggatctgggagtctcctctccttctagctgccaaagataatgatgtccaggccctgaacaagttgctcaagtatgaggattgcaaggtgcaccagagaggtaagaagcacaaatgcagcatgatctcctaggtgagccccacacatggggcctcccaggagtgcccaggacctcgtgctgttggcctctgaatctatcgtctccaatccgctgtcccacagaagccatataacccacctctctgtaaatgccaggagccatgggggaaacagcgctacacatagcagccctctatgacaacctggaggccgccatggtgctgatggaggctgccccggagctggtctttgagcccatgacatctgagctctatgagggtgagggcccacgggtctggggtgaagagcaggagtgactggttgggtatttcaagtcagtctctgtgatggataatttgggaaagacacaggggatctgagcctcctactctttttttctcttctctgtctcccttccgtgtcagtcctgactgcccatcactagaacgcctgccccctgaaatgccaggggcctagagaagaggaagagatgggcagcagctggatcccctgggaatcctgaacacccgagagctccctgttctccatcccaggctacccctgagggaaagagactggggtgcatatgggagggaccccctgcaggatcctggggacagacccgtgactgacagctgtctctgggccaggtcagactgcactgcacatcgctgttgtgaaccagaacatgaacctggtgcgagccctgcttgcccgcagggccagtgtctctgccagagccacaggcactgccttccgccgtagtccctgcaacctcatctactttggtgagagcagggctgggcttggaggacgggcagttggaaaggtgggcaaggcagggcagggccaggcagaggaggatcctgtcttcagccgtatctgttgggcagctgggaggagcaatccttctagggcttaattagactagaggccaatttaccccacgacccttcctctggttctgcaggaaaagtgtcctcaagccctgagctgagatgtgggggaagataaggctgtcacttgggggagactgtccaccccatcctgccatcctgcactctcctaccatagatctctctgtgtccacaggggagcaccctttgtcctttgctgcctgtgtgaacagtgaggagatcgtgcggctgctcattgagcatggagctgacatccgggcccaggactccctgggtaagagctgagatggggaggggagctgggatgctgcagggagtgagggacagggtgaggagaggggctgggaccttcaggaagacctcagggtggggatggggacatcagggactttaggccagtggccacatgataccctgtgtcctccccaggaaacacagtgttacacatcctcatcctccagcccaacaaaacctttgcctgccagatgtacaacctgttgctgtcctacgacagacatggggaccacctgcagcccctggacctcgtgcccaatcaccagggtctcacccctttcaagctggctggagtggagggtaacactgtggtgagagacggtccccatccctgaggtgtctttctaatgaccctcaacctatcccgctggccctgggagaaacagaggtgaacgcgatccctgatgcttagatcccattctcaactcagaaatttttcaacccctcccactgtggttacctgttccctttcttgcccactccttttcccctgaggcattgggggttacagagtctagatcccatgctaggattgtctgtaatgccccagcccaccttccctttcagcccccagagcagggccctccagcctctcgtctctcctttccaaactctggagggagtcatgggagaggatgaggaacctatgaatgtcactgtgaatgtgggttcttctgccctctaaaggctgtcatcaaaatgaaagggcagccaccttctccaggggtgccgtcctcctgcacatgcatcctatccacactctgtgaccgtcccctttgcttactgctcctgagtcatcttcactttcccttagatgtttcagcacctgatgcagaagcggaagcacacccagtggacgtatggaccactgacctcgactctctatgacctcacagagatcgactcctcaggggatgagcagtccctgctggaacttatcatcaccaccaagaagcgggaggtatggctcatgacagcaggctgtggctggggaggggtgtcagggtctctgagccacctgttctctttctgttgcaggctcgccagatcctggaccagacgccggtgaaggagctggtgagcctcaagtggaagcggtacgggcggccgtacttctgcatgctgggtgccatatatctgctgtacatcatctgcttcaccatgtgctgcatctaccgccccctcaagcccaggaccaataaccgcacgagcccccgggacaacaccctcttacagcagaagctacttcaggtgacacccttgtaggagcagatcagcagggcaggacttggctctctgtcctcagagactggtgtccctttcctccctcacaccatttctccccttgctctaatctcaaatatatgggtacaaactccaaatgcacgcccacaaaaacacacatacgctcttactctgagagcagagtttgagaagacccaaacctaacagattaaaaagaatctgctaagactggtgaccctgggcaccatggaaatgcagggcagaggcctgaaagccctgagcattttgactgttcttctcccccattaggaagcctacatgacccctaaggacgatatccggctggtcggggagctggtgactgtcattggggctatcatcatcctgctggtagaggtgaggtgtggatggactctgggtgaggctgtctgcccgaggaatccagcccaagttccggtatctgagtgcctttgtgtctccctgacctcttcaggttccagacatcttcagaatgggggtcactcgcttctttggacagaccatccttgggggcccattccatgtcctcatgtgagtttccttcctctcactcccatcccttccctcaacagggctccagttccactccttggattcctgacctctcaagaaccttagctccagagccccctctctagtgctgtgtgtatgaccctgggcattgagtgtggggaggctgaatctgcatgtgtgggtactttcccagctacattcttgctgtcaggtccccaggatcatcccagccctcccctcatcaccctcctccctgctcccccagcatcacctatgccttcatggtgctggtgaccatggtgatgcggctcatcagtgccagcggggaggtggtacccatgtcctttgcactcgtgctgggctggtgcaacgtcatgtacttcgcccgaggattccagatgctaggccccttcaccatcatgattcagaaggtcagtcctccccccaagctccctagagaaaggccccagagccacagtcagcagacggtcccataaagggcagaacagtagacattgcaggttctgcaagccacacatggcctcactgcatgtttttcttcttttttaacaatccttttaaaaaatgtagaaacccttttcagttcaaaggccacaccaaagcaggtcaggtagatctggtccacaggccatagatagccaatccctgtcccagagggtggagctgtgagacttgtcggggtgagacctgttagaggctggatggggcaattgcttggggaatgtgtgcagatgttctctgcctcctgctccttctagatgatttttggcgacctgatgcgattctgctggctgatggctgtggtcatcctgggctttgcttcaggtaatcatctgtccaggaccaggggccatggcagggaagagatgaggaagtctagggggcactggctctggctaaacttggggaggaggagtaatgcagagatcagaggagacctatggtatcagaggatgggacgtcctccagaggtgagaaaaatcgggagtgttagggagaggtggctcttaggatcaagatgaggctcatacaaaactagggaccgtaaaaacccaaagtttggagcactgcagagctggtgatattgagatgaagggaccaggatggacatgcacgcagagcccggggtgggctggtcgtctgcatggttgccatggtaaccctcacccccttgggtggagcagccttctatatcatcttccagacagaggaccccgaggagctaggccacttctacgactaccccatggccctgttcagcaccttcgagctgttccttaccatcatcgatggcccagccaactacaacgtggacctgcccttcatgtacagcatcacctatgctgcctttgccatcatcgccacactgctcatgctcaacctcctcattgccatgatgggcgacactcactggcgagtggcccatgagcgggatgagctgtggagggcccaggtgagccccctggtggcagggagggttagggcaagtcatccccttcctaccaaggaacctgccaagctgagagacaggatatctccaccccacttatgtttggacagttgtggcaaagctagcaaaatcatgcaaaatgtacagaagcactgattagcaattcaaccaggcaatactggaatcgctgagaagaatgcctcacagttttctcaacagttaaaagctcagtgttttctagaggaatcaacaagaaataaatcaaaagaaaattaacgttggctaaaattgcactcagtacattttgttcccaaataaaaactggagtatcaagtcttcttgataatatttaagtctgcaaaatttgatatggaaagcaggatgtgttaaaaaagtaatgccaccaaaacttcctatagtagcagaagctatcttcagccagatcttcaagatagggagagaagaccatgagatgaatcaaatcctcatttaaaaaacacctagaaaataatttatctaaaaaaatcatttcagcaaaataatggaaatttcccaaactggaaggcatttaactatgctgtgtagaaaacggagtggaaaaactaagctgggaaataaggttcactcagaaaaatattttctccaggaatatatattgatattctaagtgggatgtttatatttataagtggcctttatgtctgtagggtcaaaatatctgggagcccttaaaagccctttctatttgctttctctggtgcctgtgctcctgggaatggggcttctgcttcctgtctttctcctgcctctggcctggctgcgtcatggatgttgggtcattgggtaaagaattgttggtctcaagctctatcaactctctcccactgaagaaggtcaacaaaggctgccctacccctacctctgtctgcgcccagcctcatctctgacttctccttttgttcccatacgcagattgtggccaccacagtgatgctggagcggaagctgcctcgctgcctgtggcctcgctccgggatctgcggacgggagtatggcctgggagaccgctggttcctgcggtgagtgatatgcgggggtaggtgtcccctgagaagcctcatcggcagggtatccccctgctcagacagcttccggctcctgggttccctgtggaggcctgtgtgctccctaggctctatgcttgttgattgagctggtgaggaaggggtcccgtttggagctcagacttcccaaagcatccagggagtctgtggcagagcctgctgctttctgaggcctagctgccaaggggccagtgacccaggcatccaccatggctgcagaaaagggaaaaggccagcaatggcggggatgggaggaccaggggataacagacaagcatccttcttggatctgttcttcaagtcctggctgtgtctcaagtcctcccgcattccacagggtggaagacaggcaagatctcaaccggcagcggatccaacgctacgcacaggccttccacacccggggctctgaggatttggacaaagactcagtggaaaaactagagctgggctgtcccttcagcccccacctgtcccttcctatgccctcagtgtctcgaagtacctcccgcagcagtgccaattgggaaaggcttcggcaagggaccctgaggagagacctgcgtgggataatcaacaggggtctggaggacggggagagctgggaatatcagatctgactgcgtgttctcacttcgcttcctggaacttgctctcattttcctgggtgcatcaaacaaaacaaaaaccaaacacccagaggtctcatctcccaggccccaggggagaaagaggagtagcatgaacgccaaggaatgtacgttgagaatcactgctccaggcctgcattactccttcagctctggggcagaggaagcccagcccaagcacggggctggcagggcgtgaggaactctcctgtggcctgctcatcacccttccgacaggagcactgcatgtcagagcactttaaaaacaggccagcctgcttgggcgctcggtctccaccccagggtcataagtggggagagagcccttcccagggcacccaggcaggtgcagggaagtgcagagcttgtggaaagcgtgtgagtgagggagacaggaacggctctgggggtgggaagtggggctaggtcttgccaactccatcttcaataaagtcgttttcggatccct

SEQ ID NO: 2 - protein, 765 aa, Homo sapiens
  TRPV6 (1)..(765)
MGPLQGDGGPALGGADVAPRLSPVRVWPRPQAPKEPALHPMGLSLPKEKGLILCLWSKFCRWFQRRESWAQSRDEQNLLQQKRIWESPLLLAAKDNDVQALNKLLKYEDCKVHQRGAMGETALHIAALYDNLEAAMVLMEAAPELVFEPMTSELYEGQTALHIAVVNQNMNLVRALLARRASVSARATGTAFRRSPCNLIYFGEHPLSFAACVNSEEIVRLLIEHGADIRAQDSLGNTVLHILILQPNKTFACQMYNLLLSYDRHGDHLQPLDLVPNHQGLTPFKLAGVEGNTVMFQHLMQKRKHTQWTYGPLTSTLYDLTEIDSSGDEQSLLELIITTKKREARQILDQTPVKELVSLKWKRYGRPYFCMLGAIYLLYIICFTMCCIYRPLKPRTNNRTSPRDNTLLQQKLLQEAYMTPKDDIRLVGELVTVIGAIIILLVEVPDIFRMGVTRFFGQTILGGPFHVLIITYAFMVLVTMVMRLISASGEVVPMSFALVLGWCNVMYFARGFQMLGPFTIMIQKMIFGDLMRFCWLMAVVILGFASAFYIIFQTEDPEELGHFYDYPMALFSTFELFLTIIDGPANYNVDLPFMYSITYAAFAIIATLLMLNLLIAMMGDTHWRVAHERDELWRAQIVATTVMLERKLPRCLWPRSGICGREYGLGDRWFLRVEDRQDLNRQRIQRYAQAFHTRGSEDLDKDSVEKLELGCPFSPHLSLPMPSVSRSTSRSSANWERLRQGTLRRDLRGIINRGLEDGESWEYQI

SEQ ID NO: 3 - protein, 31 aa, Homo sapiens
PLKPRTNNRTSPRDNTLLQQKLLQEAYMTPK

SEQ ID NO: 4 - protein, 13 aa, Homo sapiens
IFQTEDPEELGHF

SEQ ID NO: 5 - protein, 12 aa, Homo sapiens
DGPANYNVDLPF

SEQ ID NO: 6 - DNA, 339 bp, Mus musculus
gacattgtgatgtcacagtctccatcctccctagctgtgtcagttggagagaaggttactatgagctgcaagtccagtcagagccttttatatagtaccaatcaaaagaactacttggcctggtcccagcagaaaccagggcagtctcctaaactgctgatttactgggcatccactagggaatctggggtccctgatcgcttcacaggcagtggatctgggacagatttcactctcaccatcagcagtgtgaaggctgaagacctggcagtttattactgtcagcaatattatagctatccgtggacgttcggtggaggcaccaagctggaaatcaaa

SEQ ID NO: 7 - protein, 8 aa, Mus musculus
GYTFTSYW

SEQ ID NO: 8 - protein, 8 aa, Mus musculus
IDPSDGYT

SEQ ID NO: 9 - protein, 6 aa, Mus musculus
GWAGDF

SEQ ID NO: 10 - protein, 11 aa, Mus musculus
QSLLDSDGKTY

SEQ ID NO: 11 - protein, 4 aa, Mus musculus
  misc_feature (4)..(4): Xaa is absent.
LVSX

SEQ ID NO: 12 - protein, 9 aa, Mus musculus
WQGTHFPQT

SEQ ID NO: 13 - protein, 8 aa, Mus musculus
GFTFSYYW

SEQ ID NO: 14 - protein, 10 aa, Mus musculus
IRLKSHNYAT

SEQ ID NO: 15 - protein, 16 aa, Mus musculus
ARLAYDGERYYYALDY

SEQ ID NO: 16 - protein, 12 aa, Mus musculus
QSLLYSNNQKNY

SEQ ID NO: 17 - protein, 4 aa, Mus musculus
  misc_feature (4)..(4): Xaa is absent.
WASX

SEQ ID NO: 18 - protein, 9 aa, Mus musculus
QQYYSYPFT

SEQ ID NO: 19 - protein, 8 aa, Mus musculus
AFTFSHYW

SEQ ID NO: 20 - protein, 10 aa, Mus musculus
IRLKSYNYAT

SEQ ID NO: 21 - protein, 15 aa, Mus musculus
TRLGYFGSLYYAMDY

SEQ ID NO: 22 - protein, 12 aa, Mus musculus
QSLLYSTNQKNY

SEQ ID NO: 23 - protein, 4 aa, Mus musculus
  misc_feature (4)..(4): Xaa is absent.
WASX

SEQ ID NO: 24 - protein, 9 aa, Mus musculus
QQYYSYPWT

SEQ ID NO: 25 - protein, 113 aa, Mus musculus
QVQVQQPGAELVKPGTSVKLSCKASGYTFTSYWMHWVKQRPGQGLEWIGEIDPSDGYTNYNQKFRGKATLSVDKSSTTAYMQLSSLTSEDSAVYYCGWAGDFWGQGTTLTVSS

SEQ ID NO: 26 - protein, 112 aa, Mus musculus
DVVLTQSPLTLSVTIGQPASISCKSSQSLLDSDGKTYLNWLLQRPGQSPKRLIYLVSKLDSAAPDRFAGSGSGTDFTLKISRVEAEDLGIYYCWQGTHFPQTFGGGTKLEIK

SEQ ID NO: 27 - protein, 125 aa, Mus musculus
EVKLEESGGGLVQPGGSMKLSCVASGFTFSYYWMNWVRQSPEKGLEWVAEIRLKSHNYATHYAESVKGRFTISRDDSKSSVYLQMNNLRSEDTGIYYCARLAYDGERYYYALDYWGQGTSVTVSS

SEQ ID NO: 28 - protein, 113 aa, Mus musculus
DIVMSQSPSSLAVSVGEKFTMSCKSSQSLLYSNNQKNYLAWYQQKPGQSPKLLIYWASTRESGVPDRFTGSGYGTDFTLTISSVKAEDLAVYYCQQYYSYPFTFGSGTKLEIK

SEQ ID NO: 29 - protein, 124 aa, Mus musculus
EVMLEESGGGLVQPGGSMKLSCVASAFTFSHYWMNWVRQSPEKGLEWVAEIRLKSYNYATHYAESVKGRFTISRDDSKSSVYLQMNSLRPEDTGIYYCTRLGYFGSLYYAMDYWGQGTSVTVSS

SEQ ID NO: 30 - protein, 112 aa, Mus musculus
DIVMSQSPSSLAVSVGEKVTMSCKSSQSLLYSTNQKNYLAWSQQKPGQSPKLLIYWASTESGVPDRFTGSGSGTDFTLTISSVKAEDLAVYYCQQYYSYPWTFGGGTKLEIK

SEQ ID NO: 31 - DNA, 339 bp, Mus musculus
caggtccaagtgcagcagcctggggctgagcttgtgaagcctgggacttcagtgaagctgtcctgcaaggcttctggctacaccttcaccagctactggatgcactgggtgaagcagaggcctggacaaggccttgagtggatcggagagattgatccttctgatggttatactaactacaatcaaaagttcaggggcaaggccacattgtctgtagacaaatcctccaccacagcctacatgcagctcagcagcctgacatctgaggactctgcggtctattactgtgggtgggcgggggacttctggggccaaggcaccactctcacagtctcctca

SEQ ID NO: 32 - DNA, 336 bp, Mus musculus
gatgttgtgctgacccagagtccactcactttgtcggttaccattggacaaccagcctccatctcttgcaagtcaagtcagagcctcttagatagtgatggaaagacatatttgaattggttgttacagaggccaggccagtctccaaagcgcctaatctatctggtgtctaagctggactctgcagcccctgacaggttcgctggcagtggatcagggacagatttcacactgaaaatcagcagagtggaggctgaagatttgggaatttactattgctggcaaggtacacattttcctcagacgttcggtggaggcaccaagctggaaatcaaa

SEQ ID NO: 33 - DNA, 375 bp, Mus musculus
gaagtgaagcttgaggagtctggaggaggcttggtgcaacctggaggatccatgaaactctcctgtgttgcctctggattcactttcagttactactggatgaactgggtccgccagtctccagagaaggggcttgagtgggttgctgaaattagattgaaatctcataattatgcaacacattatgcggagtctgtgaaagggaggttcaccatctcaagagatgattccaaaagtagtgtctacctgcaaatgaacaacttaagatctgaagacactggcatttattactgtgccaggcttgcttacgacggggagcggtattactatgctctggactactggggtcaaggaacctcagtcaccgtctcctca

SEQ ID NO: 34 - DNA, 339 bp, Mus musculus
gacattgtgatgtcacagtctccatcctccctagctgtgtcagttggagagaagtttactatgagctgcaagtccagtcagagccttttatatagtaacaatcaaaagaactacttggcctggtaccagcagaaaccagggcagtctcctaaactgctgatttactgggcatccactagggaatctggggtccctgatcgcttcacaggcagtggatatgggacagatttcactctcaccatcagcagtgtgaaggctgaagacctggcagtttattactgtcagcaatattatagctatccattcacgttcggctcggggacaaagttggaaataaaa

SEQ ID NO: 35 - DNA, 372 bp, Mus musculus
gaagtgatgcttgaggagtctggaggaggcttagtgcaacctggaggatccatgaagctctcctgtgttgcctctgcattcactttcagtcactactggatgaactgggtccgccagtctccagagaaggggcttgagtgggttgctgaaattagattgaaatcttataattatgcaacacattatgcggagtctgtgaaagggaggttcaccatctccagagatgattccaagagtagtgtctacctgcaaatgaacagcctaaggcctgaagacactggcatttattactgtaccaggcttggttacttcggtagcctctactatgctatggactactggggtcaaggaacctcagtcaccgtctcctca